European Patent Application EP 4 286 408 A1, published December 6, 2023. Title: Bi or Multi-Specific Antibody. Applicant: Samsung Biologics. The sequence listing filed with the application follows.

SEQUENCE LISTING (68 sequences)

SEQ ID NO: 1 - protein, 123 aa, Artificial Sequence [sequence omitted]

SEQ ID NO: 2 - protein, 107 aa, Artificial Sequence [sequence omitted]

SEQ ID NO: 3 - protein, 120 aa, Artificial Sequence [sequence omitted]

SEQ ID NO: 4 - protein, 107 aa, Artificial Sequence [sequence omitted]

SEQ ID NO: 5 - protein, 98 aa, Artificial Sequence
  IgG1 CH1
ASTKGPSVFPLAPSSKSTSGGTAALGCLVKDYFPEPVTVSWNSGALTSGVHTFPAVLQSSGLYSLSSVVTVPSSSLGTQTYICNVNHKPSNTKVDKKV

SEQ ID NO: 6 - protein, 110 aa, Artificial Sequence
  IgG1 CH2
APELLGGPSVFLFPPKPKDTLMISRTPEVTCVVVDVSHEDPEVKFNWYVDGVEVHNAKTKPREEQYNSTYRVVSVLTVLHQDWLNGKEYKCKVSNKALPAPIEKTISKAK

SEQ ID NO: 7 - protein, 107 aa, Artificial Sequence
  IgG1 CH3
GQPREPQVYTLPPSRDELTKNQVSLTCLVKGFYPSDIAVEWESNGQPENNYKTTPPVLDSDGSFFLYSKLTVDKSRWQQGNVFSCSVMHEALHNHYTQKSLSLSPGK

SEQ ID NO: 8 - protein, 107 aa, Artificial Sequence
  IgG1 CH3-Knob
GQPREPQVYTLPPSREEMTKNQVSLWCLVKGFYPSDIAVEWESNGQPENNYKTTPPVLDSDGSFFLYSKLTVDKSRWQQGNVFSCSVMHEALHNHYTQKSLSLSPGK

SEQ ID NO: 9 - protein, 107 aa, Artificial Sequence
  IgG1 CH3-Hole
GQPREPQVYTLPPSREEMTKNQVSLSCAVKGFYPSDIAVEWESNGQPENNYKTTPPVLDSDGSFFLVSKLTVDKSRWQQGNVFSCSVMHEALHNHYTQKSLSLSPGK

SEQ ID NO: 10 - protein, 107 aa, Artificial Sequence
  IgG1 CH3-Knob S354C
GQPREPQVYTLPPCREEMTKNQVSLWCLVKGFYPSDIAVEWESNGQPENNYKTTPPVLDSDGSFFLYSKLTVDKSRWQQGNVFSCSVMHEALHNHYTQKSLSLSPGK

SEQ ID NO: 11 - protein, 107 aa, Artificial Sequence
  IgG1 CH3-Hole Y349C
GQPREPQVCTLPPSREEMTKNQVSLSCAVKGFYPSDIAVEWESNGQPENNYKTTPPVLDSDGSFFLVSKLTVDKSRWQQGNVFSCSVMHEALHNHYTQKSLSLSPGK

SEQ ID NO: 12 - protein, 107 aa, Artificial Sequence
  IgG1 CH3-Knob Y349C
GQPREPQVCTLPPSREEMTKNQVSLWCLVKGFYPSDIAVEWESNGQPENNYKTTPPVLDSDGSFFLYSKLTVDKSRWQQGNVFSCSVMHEALHNHYTQKSLSLSPGK

SEQ ID NO: 13 - protein, 107 aa, Artificial Sequence
  IgG1 CH3-Hole S354C
GQPREPQVYTLPPCREEMTKNQVSLSCAVKGFYPSDIAVEWESNGQPENNYKTTPPVLDSDGSFFLVSKLTVDKSRWQQGNVFSCSVMHEALHNHYTQKSLSLSPGK

SEQ ID NO: 14 - protein, 107 aa, Artificial Sequence [sequence omitted]

SEQ ID NO: 15 - protein, 107 aa, Artificial Sequence
  CL-Kappa-C214S
RTVAAPSVFIFPPSDEQLKSGTASVVCLLNNFYPREAKVQWKVDNALQSGNSQESVTEQDSKDSTYSLSSTLTLSKADYEKHKVYACEVTHQGLSSPVTKSFNRGES

SEQ ID NO: 16 - protein, 106 aa, Artificial Sequence
  CL-Lambda
GQPKANPTVTLFPPSSEELQANKATLVCLISDFYPGAVTVAWKADGSPVKAGVETTKPSKQSNNKYAASSYLSLTPEQWKSHRSYSCQVTHEGSTVEKTVAPTECS

SEQ ID NO: 17 - protein, 106 aa, Artificial Sequence
  CL-Lambda-C214S
GQPKANPTVTLFPPSSEELQANKATLVCLISDFYPGAVTVAWKADGSPVKAGVETTKPSKQSNNKYAASSYLSLTPEQWKSHRSYSCQVTHEGSTVEKTVAPTESS

SEQ ID NO: 18 - protein, 98 aa, Artificial Sequence
  IgG4 CH1
ASTKGPSVFPLAPCSRSTSESTAALGCLVKDYFPEPVTVSWNSGALTSGVHTFPAVLQSSGLYSLSSVVTVPSSSLGTKTYTCNVDHKPSNTKVDKRV

SEQ ID NO: 19 - protein, 98 aa, Artificial Sequence
  IgG4 CH1 C131S
ASTKGPSVFPLAPSSRSTSESTAALGCLVKDYFPEPVTVSWNSGALTSGVHTFPAVLQSSGLYSLSSVVTVPSSSLGTKTYTCNVDHKPSNTKVDKRV

SEQ ID NO: 20 - protein, 98 aa, Artificial Sequence
  IgD CH1
APTKAPDVFPIISGCRHPKDNSPVVLACLITGYHPTSVTVTWYMGTQSQPQRTFPEIQRRDSYYMTSSQLSTPLQQWRQGEYKCVVQHTASKSKKEIF

SEQ ID NO: 21 - protein, 15 aa, Artificial Sequence
  IgG1 Hinge wild type
EPKSCDKTHTCPPCP

SEQ ID NO: 22 - protein, 10 aa, Artificial Sequence
  IgG1 Hinge del EPKSC
DKTHTCPPCP

SEQ ID NO: 23 - protein, 15 aa, Artificial Sequence
  IgG1 Hinge EPKSS
EPKSSDKTHTCPPCP

SEQ ID NO: 24 - protein, 12 aa, Artificial Sequence
  IgG4 Hinge
ESKYGPPCPPCP

SEQ ID NO: 25 - protein, 2 aa, Artificial Sequence
  Elbow sequence 1
AS

SEQ ID NO: 26 - protein, 2 aa, Artificial Sequence
  Elbow sequence 2
RT

SEQ ID NO: 27 - protein, 5 aa, Artificial Sequence
  Linker1
GGGGS

SEQ ID NO: 28 - protein, 10 aa, Artificial Sequence
  Linker2
GGGGSGGGGS

SEQ ID NO: 29 - protein, 15 aa, Artificial Sequence
  Linker3
GGGGSGGGGSGGGGS

SEQ ID NO: 30 - protein, 20 aa, Artificial Sequence
  Linker4
GGGGSGGGGSGGGGSGGGGS

SEQ ID NO: 31 - protein, 562 aa, Artificial Sequence
  Q-SBL1 HC first arm
EVQLVESGGGLVQPGGSLRLSCAASGFNIKDTYIHWVRQAPGKGLEWVARIYPTNGYTRYADSVKGRFTISADTSKNTAYLQMNSLRAEDTAVYYCSRWGGDGFYAMDYWGQGTLVTVSSASPREPQVCTLPPSREEMTKNQVSLSCAVKGFYPSDIAVEWESNGQPENNYKTTPPVLDSDGSFFLVSKLTVDKSRWQQGNVFSCSVMHEALHNHYTQKSLSLSPGKGGGGSGGGGSASTKGPSVFPLAPSSKSTSGGTAALGCLVKDYFPEPVTVSWNSGALTSGVHTFPAVLQSSGLYSLSSVVTVPSSSLGTQTYICNVNHKPSNTKVDKKVDKTHTCPPCPAPELLGGPSVFLFPPKPKDTLMISRTPEVTCVVVDVSHEDPEVKFNWYVDGVEVHNAKTKPREEQYNSTYRVVSVLTVLHQDWLNGKEYKCKVSNKALPAPIEKTISKAKGQPREPQVYTLPPSREEMTKNQVSLSCAVKGFYPSDIAVEWESNGQPENNYKTTPPVLDSDGSFFLVSKLTVDKSRWQQGNVFSCSVMHEALHNHYTQKSLSLSPGK

SEQ ID NO: 32 - protein, 331 aa, Artificial Sequence
  Q-SBL1 LC first arm
DIQMTQSPSSLSASVGDRVTITCRASQDVNTAVAWYQQKPGKAPKLLIYSASFLYSGVPSRFSGSRSGTDFTLTISSLQPEDFATYYCQQHYTTPPTFGQGTKVEIKRTPREPQVYTLPPCREEMTKNQVSLWCLVKGFYPSDIAVEWESNGQPENNYKTTPPVLDSDGSFFLYSKLTVDKSRWQQGNVFSCSVMHEALHNHYTQKSLSLSPGKGGGGSGGGGSRTVAAPSVFIFPPSDEQLKSGTASVVCLLNNFYPREAKVQWKVDNALQSGNSQESVTEQDSKDSTYSLSSTLTLSKADYEKHKVYACEVTHQGLSSPVTKSFNRGES

SEQ ID NO: 33 - protein, 557 aa, Artificial Sequence
  Q-SBL2 HC first arm
EVQLVESGGGLVQPGGSLRLSCAASGFNIKDTYIHWVRQAPGKGLEWVARIYPTNGYTRYADSVKGRFTISADTSKNTAYLQMNSLRAEDTAVYYCSRWGGDGFYAMDYWGQGTLVTVSSASPREPQVCTLPPSREEMTKNQVSLSCAVKGFYPSDIAVEWESNGQPENNYKTTPPVLDSDGSFFLVSKLTVDKSRWQQGNVFSCSVMHEALHNHYTQKSLSLSPGKGGGGSASTKGPSVFPLAPSSKSTSGGTAALGCLVKDYFPEPVTVSWNSGALTSGVHTFPAVLQSSGLYSLSSVVTVPSSSLGTQTYICNVNHKPSNTKVDKKVDKTHTCPPCPAPELLGGPSVFLFPPKPKDTLMISRTPEVTCVVVDVSHEDPEVKFNWYVDGVEVHNAKTKPREEQYNSTYRVVSVLTVLHQDWLNGKEYKCKVSNKALPAPIEKTISKAKGQPREPQVYTLPPSREEMTKNQVSLSCAVKGFYPSDIAVEWESNGQPENNYKTTPPVLDSDGSFFLVSKLTVDKSRWQQGNVFSCSVMHEALHNHYTQKSLSLSPGK

SEQ ID NO: 34 - protein, 326 aa, Artificial Sequence
  Q-SBL2 LC first arm
DIQMTQSPSSLSASVGDRVTITCRASQDVNTAVAWYQQKPGKAPKLLIYSASFLYSGVPSRFSGSRSGTDFTLTISSLQPEDFATYYCQQHYTTPPTFGQGTKVEIKRTPREPQVYTLPPCREEMTKNQVSLWCLVKGFYPSDIAVEWESNGQPENNYKTTPPVLDSDGSFFLYSKLTVDKSRWQQGNVFSCSVMHEALHNHYTQKSLSLSPGKGGGGSRTVAAPSVFIFPPSDEQLKSGTASVVCLLNNFYPREAKVQWKVDNALQSGNSQESVTEQDSKDSTYSLSSTLTLSKADYEKHKVYACEVTHQGLSSPVTKSFNRGES

SEQ ID NO: 35 - protein, 567 aa, Artificial Sequence
  Q-SBL3 HC first arm
EVQLVESGGGLVQPGGSLRLSCAASGFNIKDTYIHWVRQAPGKGLEWVARIYPTNGYTRYADSVKGRFTISADTSKNTAYLQMNSLRAEDTAVYYCSRWGGDGFYAMDYWGQGTLVTVSSASPREPQVCTLPPSREEMTKNQVSLSCAVKGFYPSDIAVEWESNGQPENNYKTTPPVLDSDGSFFLVSKLTVDKSRWQQGNVFSCSVMHEALHNHYTQKSLSLSPGKGGGGSGGGGSGGGGSASTKGPSVFPLAPSSKSTSGGTAALGCLVKDYFPEPVTVSWNSGALTSGVHTFPAVLQSSGLYSLSSVVTVPSSSLGTQTYICNVNHKPSNTKVDKKVDKTHTCPPCPAPELLGGPSVFLFPPKPKDTLMISRTPEVTCVVVDVSHEDPEVKFNWYVDGVEVHNAKTKPREEQYNSTYRVVSVLTVLHQDWLNGKEYKCKVSNKALPAPIEKTISKAKGQPREPQVYTLPPSREEMTKNQVSLSCAVKGFYPSDIAVEWESNGQPENNYKTTPPVLDSDGSFFLVSKLTVDKSRWQQGNVFSCSVMHEALHNHYTQKSLSLSPGK

SEQ ID NO: 36 - protein, 336 aa, Artificial Sequence
  Q-SBL3 LC first arm
DIQMTQSPSSLSASVGDRVTITCRASQDVNTAVAWYQQKPGKAPKLLIYSASFLYSGVPSRFSGSRSGTDFTLTISSLQPEDFATYYCQQHYTTPPTFGQGTKVEIKRTPREPQVYTLPPCREEMTKNQVSLWCLVKGFYPSDIAVEWESNGQPENNYKTTPPVLDSDGSFFLYSKLTVDKSRWQQGNVFSCSVMHEALHNHYTQKSLSLSPGKGGGGSGGGGSGGGGSRTVAAPSVFIFPPSDEQLKSGTASVVCLLNNFYPREAKVQWKVDNALQSGNSQESVTEQDSKDSTYSLSSTLTLSKADYEKHKVYACEVTHQGLSSPVTKSFNRGES

SEQ ID NO: 37 - protein, 572 aa, Artificial Sequence
  Q-SBL4 HC first arm
EVQLVESGGGLVQPGGSLRLSCAASGFNIKDTYIHWVRQAPGKGLEWVARIYPTNGYTRYADSVKGRFTISADTSKNTAYLQMNSLRAEDTAVYYCSRWGGDGFYAMDYWGQGTLVTVSSASPREPQVCTLPPSREEMTKNQVSLSCAVKGFYPSDIAVEWESNGQPENNYKTTPPVLDSDGSFFLVSKLTVDKSRWQQGNVFSCSVMHEALHNHYTQKSLSLSPGKGGGGSGGGGSGGGGSGGGGSASTKGPSVFPLAPSSKSTSGGTAALGCLVKDYFPEPVTVSWNSGALTSGVHTFPAVLQSSGLYSLSSVVTVPSSSLGTQTYICNVNHKPSNTKVDKKVDKTHTCPPCPAPELLGGPSVFLFPPKPKDTLMISRTPEVTCVVVDVSHEDPEVKFNWYVDGVEVHNAKTKPREEQYNSTYRVVSVLTVLHQDWLNGKEYKCKVSNKALPAPIEKTISKAKGQPREPQVYTLPPSREEMTKNQVSLSCAVKGFYPSDIAVEWESNGQPENNYKTTPPVLDSDGSFFLVSKLTVDKSRWQQGNVFSCSVMHEALHNHYTQKSLSLSPGK

SEQ ID NO: 38 - protein, 341 aa, Artificial Sequence
  Q-SBL4 LC first arm
DIQMTQSPSSLSASVGDRVTITCRASQDVNTAVAWYQQKPGKAPKLLIYSASFLYSGVPSRFSGSRSGTDFTLTISSLQPEDFATYYCQQHYTTPPTFGQGTKVEIKRTPREPQVYTLPPCREEMTKNQVSLWCLVKGFYPSDIAVEWESNGQPENNYKTTPPVLDSDGSFFLYSKLTVDKSRWQQGNVFSCSVMHEALHNHYTQKSLSLSPGKGGGGSGGGGSGGGGSGGGGSRTVAAPSVFIFPPSDEQLKSGTASVVCLLNNFYPREAKVQWKVDNALQSGNSQESVTEQDSKDSTYSLSSTLTLSKADYEKHKVYACEVTHQGLSSPVTKSFNRGES

SEQ ID NO: 39 - protein, 567 aa, Artificial Sequence
  Q-SBL5 HC first arm
EVQLVESGGGLVQPGGSLRLSCAASGFNIKDTYIHWVRQAPGKGLEWVARIYPTNGYTRYADSVKGRFTISADTSKNTAYLQMNSLRAEDTAVYYCSRWGGDGFYAMDYWGQGTLVTVSSASPREPQVCTLPPSREEMTKNQVSLSCAVKGFYPSDIAVEWESNGQPENNYKTTPPVLDSDGSFFLVSKLTVDKSRWQQGNVFSCSVMHEALHNHYTQKSLSLSPGKGGGGSGGGGSASTKGPSVFPLAPSSKSTSGGTAALGCLVKDYFPEPVTVSWNSGALTSGVHTFPAVLQSSGLYSLSSVVTVPSSSLGTQTYICNVNHKPSNTKVDKKVEPKSSDKTHTCPPCPAPELLGGPSVFLFPPKPKDTLMISRTPEVTCVVVDVSHEDPEVKFNWYVDGVEVHNAKTKPREEQYNSTYRVVSVLTVLHQDWLNGKEYKCKVSNKALPAPIEKTISKAKGQPREPQVYTLPPSREEMTKNQVSLSCAVKGFYPSDIAVEWESNGQPENNYKTTPPVLDSDGSFFLVSKLTVDKSRWQQGNVFSCSVMHEALHNHYTQKSLSLSPGK

SEQ ID NO: 40 - protein, 331 aa, Artificial Sequence; identical to SEQ ID NO: 32
  Q-SBL5 LC first arm

SEQ ID NO: 41 - protein, 562 aa, Artificial Sequence
  Q-SBL6 HC first arm
EVQLVESGGGLVQPGGSLRLSCAASGFNIKDTYIHWVRQAPGKGLEWVARIYPTNGYTRYADSVKGRFTISADTSKNTAYLQMNSLRAEDTAVYYCSRWGGDGFYAMDYWGQGTLVTVSSASPREPQVYTLPPCREEMTKNQVSLWCLVKGFYPSDIAVEWESNGQPENNYKTTPPVLDSDGSFFLYSKLTVDKSRWQQGNVFSCSVMHEALHNHYTQKSLSLSPGKGGGGSGGGGSASTKGPSVFPLAPSSKSTSGGTAALGCLVKDYFPEPVTVSWNSGALTSGVHTFPAVLQSSGLYSLSSVVTVPSSSLGTQTYICNVNHKPSNTKVDKKVDKTHTCPPCPAPELLGGPSVFLFPPKPKDTLMISRTPEVTCVVVDVSHEDPEVKFNWYVDGVEVHNAKTKPREEQYNSTYRVVSVLTVLHQDWLNGKEYKCKVSNKALPAPIEKTISKAKGQPREPQVYTLPPSREEMTKNQVSLSCAVKGFYPSDIAVEWESNGQPENNYKTTPPVLDSDGSFFLVSKLTVDKSRWQQGNVFSCSVMHEALHNHYTQKSLSLSPGK

SEQ ID NO: 42 - protein, 331 aa, Artificial Sequence
  Q-SBL6 LC first arm
DIQMTQSPSSLSASVGDRVTITCRASQDVNTAVAWYQQKPGKAPKLLIYSASFLYSGVPSRFSGSRSGTDFTLTISSLQPEDFATYYCQQHYTTPPTFGQGTKVEIKRTPREPQVCTLPPSREEMTKNQVSLSCAVKGFYPSDIAVEWESNGQPENNYKTTPPVLDSDGSFFLVSKLTVDKSRWQQGNVFSCSVMHEALHNHYTQKSLSLSPGKGGGGSGGGGSRTVAAPSVFIFPPSDEQLKSGTASVVCLLNNFYPREAKVQWKVDNALQSGNSQESVTEQDSKDSTYSLSSTLTLSKADYEKHKVYACEVTHQGLSSPVTKSFNRGES

SEQ ID NO: 43 - protein, 562 aa, Artificial Sequence
  Q-SBL7 HC first arm
EVQLVESGGGLVQPGGSLRLSCAASGFNIKDTYIHWVRQAPGKGLEWVARIYPTNGYTRYADSVKGRFTISADTSKNTAYLQMNSLRAEDTAVYYCSRWGGDGFYAMDYWGQGTLVTVSSASPREPQVCTLPPSREEMTKNQVSLSCAVKGFYPSDIAVEWESNGQPENNYKTTPPVLDSDGSFFLVSKLTVDKSRWQQGNVFSCSVMHEALHNHYTQKSLSLSPGKGGGGSGGGGSASTKGPSVFPLAPSSKSTSGGTAALGCLVKDYFPEPVTVSWNSGALTSGVHTFPAVLQSSGLYSLSSVVTVPSSSLGTQTYICNVNHKPSNTKVDKKVDKTHTCPPCPAPELLGGPSVFLFPPKPKDTLMISRTPEVTCVVVDVSHEDPEVKFNWYVDGVEVHNAKTKPREEQYNSTYRVVSVLTVLHQDWLNGKEYKCKVSNKALPAPIEKTISKAKGQPREPQVYTLPPSREEMTKNQVSLWCLVKGFYPSDIAVEWESNGQPENNYKTTPPVLDSDGSFFLYSKLTVDKSRWQQGNVFSCSVMHEALHNHYTQKSLSLSPGK

SEQ ID NO: 44 - protein, 331 aa, Artificial Sequence; identical to SEQ ID NO: 32
  Q-SBL7 LC first arm

SEQ ID NO: 45 - protein, 562 aa, Artificial Sequence
  Q-SBL8 HC first arm
EVQLVESGGGLVQPGGSLRLSCAASGFNIKDTYIHWVRQAPGKGLEWVARIYPTNGYTRYADSVKGRFTISADTSKNTAYLQMNSLRAEDTAVYYCSRWGGDGFYAMDYWGQGTLVTVSSASPREPQVYTLPPCREEMTKNQVSLWCLVKGFYPSDIAVEWESNGQPENNYKTTPPVLDSDGSFFLYSKLTVDKSRWQQGNVFSCSVMHEALHNHYTQKSLSLSPGKGGGGSGGGGSASTKGPSVFPLAPSSKSTSGGTAALGCLVKDYFPEPVTVSWNSGALTSGVHTFPAVLQSSGLYSLSSVVTVPSSSLGTQTYICNVNHKPSNTKVDKKVDKTHTCPPCPAPELLGGPSVFLFPPKPKDTLMISRTPEVTCVVVDVSHEDPEVKFNWYVDGVEVHNAKTKPREEQYNSTYRVVSVLTVLHQDWLNGKEYKCKVSNKALPAPIEKTISKAKGQPREPQVYTLPPSREEMTKNQVSLWCLVKGFYPSDIAVEWESNGQPENNYKTTPPVLDSDGSFFLYSKLTVDKSRWQQGNVFSCSVMHEALHNHYTQKSLSLSPGK

SEQ ID NO: 46 - protein, 331 aa, Artificial Sequence; identical to SEQ ID NO: 42
  Q-SBL8 LC first arm

SEQ ID NO: 47 - protein, 562 aa, Artificial Sequence
  Q-SBL9 HC first arm
EVQLVESGGGLVQPGGSLRLSCAASGFNIKDTYIHWVRQAPGKGLEWVARIYPTNGYTRYADSVKGRFTISADTSKNTAYLQMNSLRAEDTAVYYCSRWGGDGFYAMDYWGQGTLVTVSSASPREPQVYTLPPCREEMTKNQVSLSCAVKGFYPSDIAVEWESNGQPENNYKTTPPVLDSDGSFFLVSKLTVDKSRWQQGNVFSCSVMHEALHNHYTQKSLSLSPGKGGGGSASTKGPSVFPLAPSSKSTSGGTAALGCLVKDYFPEPVTVSWNSGALTSGVHTFPAVLQSSGLYSLSSVVTVPSSSLGTQTYICNVNHKPSNTKVDKKVEPKSSDKTHTCPPCPAPELLGGPSVFLFPPKPKDTLMISRTPEVTCVVVDVSHEDPEVKFNWYVDGVEVHNAKTKPREEQYNSTYRVVSVLTVLHQDWLNGKEYKCKVSNKALPAPIEKTISKAKGQPREPQVCTLPPSREEMTKNQVSLSCAVKGFYPSDIAVEWESNGQPENNYKTTPPVLDSDGSFFLVSKLTVDKSRWQQGNVFSCSVMHEALHNHYTQKSLSLSPGK

SEQ ID NO: 48 - protein, 326 aa, Artificial Sequence
  Q-SBL9 LC first arm
DIQMTQSPSSLSASVGDRVTITCRASQDVNTAVAWYQQKPGKAPKLLIYSASFLYSGVPSRFSGSRSGTDFTLTISSLQPEDFATYYCQQHYTTPPTFGQGTKVEIKRTPREPQVCTLPPSREEMTKNQVSLWCLVKGFYPSDIAVEWESNGQPENNYKTTPPVLDSDGSFFLYSKLTVDKSRWQQGNVFSCSVMHEALHNHYTQKSLSLSPGKGGGGSRTVAAPSVFIFPPSDEQLKSGTASVVCLLNNFYPREAKVQWKVDNALQSGNSQESVTEQDSKDSTYSLSSTLTLSKADYEKHKVYACEVTHQGLSSPVTKSFNRGES

SEQ ID NO: 49 - protein, 562 aa, Artificial Sequence
  R-SBL1 HC first arm
EVQLVESGGGLVQPGGSLRLSCAASGFNIKDTYIHWVRQAPGKGLEWVARIYPTNGYTRYADSVKGRFTISADTSKNTAYLQMNSLRAEDTAVYYCSRWGGDGFYAMDYWGQGTLVTVSSASPREPQVCTLPPSREEMTKNQVSLSCAVKGFYPSDIAVEWESNGQPENNYKTTPPVLDSDGSFFLVSKLTVDKSRWQQGNVFSCSVMHEALHNHYTQKSLSLSPGKGGGGSGGGGSASTKGPSVFPLAPSSRSTSESTAALGCLVKDYFPEPVTVSWNSGALTSGVHTFPAVLQSSGLYSLSSVVTVPSSSLGTKTYTCNVDHKPSNTKVDKRVDKTHTCPPCPAPELLGGPSVFLFPPKPKDTLMISRTPEVTCVVVDVSHEDPEVKFNWYVDGVEVHNAKTKPREEQYNSTYRVVSVLTVLHQDWLNGKEYKCKVSNKALPAPIEKTISKAKGQPREPQVYTLPPSREEMTKNQVSLSCAVKGFYPSDIAVEWESNGQPENNYKTTPPVLDSDGSFFLVSKLTVDKSRWQQGNVFSCSVMHEALHNHYTQKSLSLSPGK

SEQ ID NO: 50 - protein, 331 aa, Artificial Sequence; identical to SEQ ID NO: 32
  R-SBL1 LC first arm

SEQ ID NO: 51 - protein, 557 aa, Artificial Sequence
  R-SBL2 HC first arm
EVQLVESGGGLVQPGGSLRLSCAASGFNIKDTYIHWVRQAPGKGLEWVARIYPTNGYTRYADSVKGRFTISADTSKNTAYLQMNSLRAEDTAVYYCSRWGGDGFYAMDYWGQGTLVTVSSASPREPQVCTLPPSREEMTKNQVSLSCAVKGFYPSDIAVEWESNGQPENNYKTTPPVLDSDGSFFLVSKLTVDKSRWQQGNVFSCSVMHEALHNHYTQKSLSLSPGKGGGGSASTKGPSVFPLAPSSRSTSESTAALGCLVKDYFPEPVTVSWNSGALTSGVHTFPAVLQSSGLYSLSSVVTVPSSSLGTKTYTCNVDHKPSNTKVDKRVDKTHTCPPCPAPELLGGPSVFLFPPKPKDTLMISRTPEVTCVVVDVSHEDPEVKFNWYVDGVEVHNAKTKPREEQYNSTYRVVSVLTVLHQDWLNGKEYKCKVSNKALPAPIEKTISKAKGQPREPQVYTLPPSREEMTKNQVSLSCAVKGFYPSDIAVEWESNGQPENNYKTTPPVLDSDGSFFLVSKLTVDKSRWQQGNVFSCSVMHEALHNHYTQKSLSLSPGK

SEQ ID NO: 52 - protein, 326 aa, Artificial Sequence; identical to SEQ ID NO: 34
  R-SBL2 LC first arm

SEQ ID NO: 53 - protein, 567 aa, Artificial Sequence
  R-SBL3 HC first arm
EVQLVESGGGLVQPGGSLRLSCAASGFNIKDTYIHWVRQAPGKGLEWVARIYPTNGYTRYADSVKGRFTISADTSKNTAYLQMNSLRAEDTAVYYCSRWGGDGFYAMDYWGQGTLVTVSSASPREPQVCTLPPSREEMTKNQVSLSCAVKGFYPSDIAVEWESNGQPENNYKTTPPVLDSDGSFFLVSKLTVDKSRWQQGNVFSCSVMHEALHNHYTQKSLSLSPGKGGGGSGGGGSGGGGSASTKGPSVFPLAPSSRSTSESTAALGCLVKDYFPEPVTVSWNSGALTSGVHTFPAVLQSSGLYSLSSVVTVPSSSLGTKTYTCNVDHKPSNTKVDKRVDKTHTCPPCPAPELLGGPSVFLFPPKPKDTLMISRTPEVTCVVVDVSHEDPEVKFNWYVDGVEVHNAKTKPREEQYNSTYRVVSVLTVLHQDWLNGKEYKCKVSNKALPAPIEKTISKAKGQPREPQVYTLPPSREEMTKNQVSLSCAVKGFYPSDIAVEWESNGQPENNYKTTPPVLDSDGSFFLVSKLTVDKSRWQQGNVFSCSVMHEALHNHYTQKSLSLSPGK

SEQ ID NO: 54 - protein, 336 aa, Artificial Sequence; identical to SEQ ID NO: 36
  R-SBL3 LC first arm

SEQ ID NO: 55 - protein, 572 aa, Artificial Sequence
  R-SBL4 HC first arm
EVQLVESGGGLVQPGGSLRLSCAASGFNIKDTYIHWVRQAPGKGLEWVARIYPTNGYTRYADSVKGRFTISADTSKNTAYLQMNSLRAEDTAVYYCSRWGGDGFYAMDYWGQGTLVTVSSASPREPQVCTLPPSREEMTKNQVSLSCAVKGFYPSDIAVEWESNGQPENNYKTTPPVLDSDGSFFLVSKLTVDKSRWQQGNVFSCSVMHEALHNHYTQKSLSLSPGKGGGGSGGGGSGGGGSGGGGSASTKGPSVFPLAPSSRSTSESTAALGCLVKDYFPEPVTVSWNSGALTSGVHTFPAVLQSSGLYSLSSVVTVPSSSLGTKTYTCNVDHKPSNTKVDKRVDKTHTCPPCPAPELLGGPSVFLFPPKPKDTLMISRTPEVTCVVVDVSHEDPEVKFNWYVDGVEVHNAKTKPREEQYNSTYRVVSVLTVLHQDWLNGKEYKCKVSNKALPAPIEKTISKAKGQPREPQVYTLPPSREEMTKNQVSLSCAVKGFYPSDIAVEWESNGQPENNYKTTPPVLDSDGSFFLVSKLTVDKSRWQQGNVFSCSVMHEALHNHYTQKSLSLSPGK

SEQ ID NO: 56 - protein, 341 aa, Artificial Sequence; identical to SEQ ID NO: 38
  R-SBL4 LC first arm

SEQ ID NO: 57 - protein, 567 aa, Artificial Sequence
  R-SBL5 HC first arm
EVQLVESGGGLVQPGGSLRLSCAASGFNIKDTYIHWVRQAPGKGLEWVARIYPTNGYTRYADSVKGRFTISADTSKNTAYLQMNSLRAEDTAVYYCSRWGGDGFYAMDYWGQGTLVTVSSASPREPQVCTLPPSREEMTKNQVSLSCAVKGFYPSDIAVEWESNGQPENNYKTTPPVLDSDGSFFLVSKLTVDKSRWQQGNVFSCSVMHEALHNHYTQKSLSLSPGKGGGGSGGGGSASTKGPSVFPLAPSSRSTSESTAALGCLVKDYFPEPVTVSWNSGALTSGVHTFPAVLQSSGLYSLSSVVTVPSSSLGTKTYTCNVDHKPSNTKVDKRVEPKSSDKTHTCPPCPAPELLGGPSVFLFPPKPKDTLMISRTPEVTCVVVDVSHEDPEVKFNWYVDGVEVHNAKTKPREEQYNSTYRVVSVLTVLHQDWLNGKEYKCKVSNKALPAPIEKTISKAKGQPREPQVYTLPPSREEMTKNQVSLSCAVKGFYPSDIAVEWESNGQPENNYKTTPPVLDSDGSFFLVSKLTVDKSRWQQGNVFSCSVMHEALHNHYTQKSLSLSPGK

SEQ ID NO: 58 - protein, 331 aa, Artificial Sequence; identical to SEQ ID NO: 32
  R-SBL5 LC first arm

SEQ ID NO: 59 - protein, 564 aa, Artificial Sequence
  R-SBL6 HC first arm
EVQLVESGGGLVQPGGSLRLSCAASGFNIKDTYIHWVRQAPGKGLEWVARIYPTNGYTRYADSVKGRFTISADTSKNTAYLQMNSLRAEDTAVYYCSRWGGDGFYAMDYWGQGTLVTVSSASPREPQVCTLPPSREEMTKNQVSLSCAVKGFYPSDIAVEWESNGQPENNYKTTPPVLDSDGSFFLVSKLTVDKSRWQQGNVFSCSVMHEALHNHYTQKSLSLSPGKGGGGSGGGGSASTKGPSVFPLAPSSRSTSESTAALGCLVKDYFPEPVTVSWNSGALTSGVHTFPAVLQSSGLYSLSSVVTVPSSSLGTKTYTCNVDHKPSNTKVDKRVESKYGPPCPPCPAPELLGGPSVFLFPPKPKDTLMISRTPEVTCVVVDVSHEDPEVKFNWYVDGVEVHNAKTKPREEQYNSTYRVVSVLTVLHQDWLNGKEYKCKVSNKALPAPIEKTISKAKGQPREPQVYTLPPSREEMTKNQVSLSCAVKGFYPSDIAVEWESNGQPENNYKTTPPVLDSDGSFFLVSKLTVDKSRWQQGNVFSCSVMHEALHNHYTQKSLSLSPGK

SEQ ID NO: 60 - protein, 331 aa, Artificial Sequence; identical to SEQ ID NO: 32
  R-SBL6 LC first arm

SEQ ID NO: 61 - protein, 453 aa, Artificial Sequence
  LC-1 HC second arm
EVQLVESGGGLVQPGGSLRLSCAASGYTFTNYGMNWVRQAPGKGLEWVGWINTYTGEPTYAADFKRRFTFSLDTSKSTAYLQMNSLRAEDTAVYYCAKYPHYYGSSHWYFDVWGQGTLVTVSSASTKGPSVFPLAPSSKSTSGGTAALGCLVKDYFPEPVTVSWNSGALTSGVHTFPAVLQSSGLYSLSSVVTVPSSSLGTQTYICNVNHKPSNTKVDKKVEPKSCDKTHTCPPCPAPELLGGPSVFLFPPKPKDTLMISRTPEVTCVVVDVSHEDPEVKFNWYVDGVEVHNAKTKPREEQYNSTYRVVSVLTVLHQDWLNGKEYKCKVSNKALPAPIEKTISKAKGQPREPQVYTLPPCREEMTKNQVSLWCLVKGFYPSDIAVEWESNGQPENNYKTTPPVLDSDGSFFLYSKLTVDKSRWQQGNVFSCSVMHEALHNHYTQKSLSLSPGK

SEQ ID NO: 62 - protein, 214 aa, Artificial Sequence
  LC-1 LC second arm
DIQMTQSPSSLSASVGDRVTITCSASQDISNYLNWYQQKPGKAPKVLIYFTSSLHSGVPSRFSGSGSGTDFTLTISSLQPEDFATYYCQQYSTVPWTFGQGTKVEIKRTVAAPSVFIFPPSDEQLKSGTASVVCLLNNFYPREAKVQWKVDNALQSGNSQESVTEQDSKDSTYSLSSTLTLSKADYEKHKVYACEVTHQGLSSPVTKSFNRGEC

SEQ ID NO: 63 - protein, 453 aa, Artificial Sequence
  LC-3 HC second arm
EVQLVESGGGLVQPGGSLRLSCAASGYTFTNYGMNWVRQAPGKGLEWVGWINTYTGEPTYAADFKRRFTFSLDTSKSTAYLQMNSLRAEDTAVYYCAKYPHYYGSSHWYFDVWGQGTLVTVSSASTKGPSVFPLAPSSKSTSGGTAALGCLVKDYFPEPVTVSWNSGALTSGVHTFPAVLQSSGLYSLSSVVTVPSSSLGTQTYICNVNHKPSNTKVDKKVEPKSCDKTHTCPPCPAPELLGGPSVFLFPPKPKDTLMISRTPEVTCVVVDVSHEDPEVKFNWYVDGVEVHNAKTKPREEQYNSTYRVVSVLTVLHQDWLNGKEYKCKVSNKALPAPIEKTISKAKGQPREPQVYTLPPSREEMTKNQVSLWCLVKGFYPSDIAVEWESNGQPENNYKTTPPVLDSDGSFFLYSKLTVDKSRWQQGNVFSCSVMHEALHNHYTQKSLSLSPGK

SEQ ID NO: 64 - protein, 453 aa, Artificial Sequence
  LC-3-H-K HC second arm
EVQLVESGGGLVQPGGSLRLSCAASGYTFTNYGMNWVRQAPGKGLEWVGWINTYTGEPTYAADFKRRFTFSLDTSKSTAYLQMNSLRAEDTAVYYCAKYPHYYGSSHWYFDVWGQGTLVTVSSASTKGPSVFPLAPSSKSTSGGTAALGCLVKDYFPEPVTVSWNSGALTSGVHTFPAVLQSSGLYSLSSVVTVPSSSLGTQTYICNVNHKPSNTKVDKKVEPKSCDKTHTCPPCPAPELLGGPSVFLFPPKPKDTLMISRTPEVTCVVVDVSHEDPEVKFNWYVDGVEVHNAKTKPREEQYNSTYRVVSVLTVLHQDWLNGKEYKCKVSNKALPAPIEKTISKAKGQPREPQVYTLPPSREEMTKNQVSLSCAVKGFYPSDIAVEWESNGQPENNYKTTPPVLDSDGSFFLVSKLTVDKSRWQQGNVFSCSVMHEALHNHYTQKSLSLSPGK

SEQ ID NO: 65 - protein, 19 aa, Artificial Sequence
  Signal sequence
MEWSWVFLFFLSVTTGVHS

SEQ ID NO: 66 - protein, 98 aa, Artificial Sequence
  IgG2 CH1
ASTKGPSVFPLAPCSRSTSESTAALGCLVKDYFPEPVTVSWNSGALTSGVHTFPAVLQSSGLYSLSSVVTVPSSNFGTQTYTCNVDHKPSNTKVDKTV

SEQ ID NO: 67 - protein, 105 aa, Artificial Sequence
  IgM CH1
GSASAPTLFPLVSCENSPSDTSSVAVGCLAQDFLPDSITFSWKYKNNSDISSTRGFPSVLRGGKYAATSQVLLPSKDVMQGTDEHVVCKVQHPNGNKEKNVPLPV

SEQ ID NO: 68 - protein, 104 aa, Artificial Sequence
  IgM CH3
TAIRVFAIPPSFASIFLTKSTKLTCLVTDLTTYDSVTISWTRQNGEAVKTHTNISESHPNATFSAVGEASICEDDWNSGERFTCTVTHTDLPSPLKQTISRPKG